European Patent Specification EP 4 052 572 B1, published November 26, 2025. Title: GENETICALLY MODIFIED MICE EXPRESSING CHIMERIC MAJOR HISTOCOMPATIBILITY COMPLEX (MHC) II MOLECULES. Applicant: Regeneron Pharmaceuticals, Inc. Application EP. The sequence listing filed with the application follows.

SEQUENCE LISTING (26 sequences)

SEQ ID NO: 1 - DNA, 19 bp, Artificial Sequence
  Synthetic
cagaacgccaggctgtaac

SEQ ID NO: 2 - DNA, 20 bp, Artificial Sequence
  Synthetic
ggagagcagggtcagtcaac

SEQ ID NO: 3 - DNA, 24 bp, Artificial Sequence
  Synthetic
caccgccactcacagctccttaca

SEQ ID NO: 4 - DNA, 22 bp, Artificial Sequence
  Synthetic
gtgggcaccatcttcatcattc

SEQ ID NO: 5 - DNA, 22 bp, Artificial Sequence
  Synthetic
cttcctttccagggtgtgactc

SEQ ID NO: 6 - DNA, 23 bp, Artificial Sequence
  Synthetic
aggcctgcgatcaggtggcacct

SEQ ID NO: 7 - DNA, 17 bp, Artificial Sequence
  Synthetic
tgcggccgatcttagcc

SEQ ID NO: 8 - DNA, 18 bp, Artificial Sequence
  Synthetic
ttgaccgattccttgcgg

SEQ ID NO: 9 - DNA, 21 bp, Artificial Sequence
  Synthetic
acgagcgggttcggcccattc

SEQ ID NO: 10 - DNA, 140 bp, Artificial Sequence
  Synthetic
tttgtaaacaaagtctacccagagacagatgacagacttcagctccaatgctgattggttcctcacttgggaccaaccctctcgagtaccgttcgtataatgtatgctatacgaagttatatgcatccgggtaggggagg

SEQ ID NO: 11 - DNA, 140 bp, Artificial Sequence
  Synthetic
cctcgacctgcagccctaggataacttcgtataatgtatgctatacgaacggtagagctccacaggcatttgggtgggcagggatggacggtgactgggacaatcgggatggaagagcatagaatgggagttagggaaga

SEQ ID NO: 12 - DNA, 110 bp, Artificial Sequence
  Synthetic
tgctgattggttcctcacttgggaccaaccctaagctttatctatgtcgggtgcggagaaagaggtaatgaaatggcacaaggagatcacacacccaaaccaaactcgcc

SEQ ID NO: 13 - DNA, 96 bp, Artificial Sequence
  Synthetic
cacatcagtgaggctagaataaattaaaatcgctaatatgaaaatggggatttgtacctctgagtgtgaaggctgggaagactgctttcaagggac

SEQ ID NO: 14 - DNA, 150 bp, Artificial Sequence
  Synthetic
tccatcacttcactgggtagcacagctgtaactgtccagcctgggtaccgagctcggatccactagtaacggccgccagtgtgctggaattcgcccttgatcgagctccctgggctgcaggtggtgggcgttgcgggtggggccggttaa

SEQ ID NO: 15 - DNA, 80 bp, Artificial Sequence
  Synthetic
atctccatcagaagggcaccggtataacttcgtataaggtatcctatacgaagttatatgcatggcctccgcgccgggtt

SEQ ID NO: 16 - DNA, 90 bp, Artificial Sequence
  Synthetic
ataacttcgtataaggtatcctatacgaagttatctcgagtggcttacaggtaggtgcgtgaagcttctacaagcacagttgccccctgg

SEQ ID NO: 17 - DNA, 90 bp, Artificial Sequence
  Synthetic
ctgtttcttccctaactcccattctatgctcttccatcccgaccgcggcccaatctctctccactacttcctgcctacatgtatgtaggt

SEQ ID NO: 18 - DNA, 80 bp, Artificial Sequence
  Synthetic
caaggtttcctcctatgatgcttgtgtgaaactcggggccggccagcatttaacagtacagggatgggagcacagctcac

SEQ ID NO: 19 - DNA, 80 bp, Artificial Sequence
  Synthetic
gaaagcagtcttcccagccttcacactcagaggtacaaatccccattttcatattagcgattttaatttattctagcctc

SEQ ID NO: 20 - DNA, 80 bp, Artificial Sequence
  Synthetic
tcttccctaactcccattctatgctcttccatcccgaccgcggcccaatctctctccactacttcctgcctacatgtatg

SEQ ID NO: 21 - DNA, 21 bp, Artificial Sequence
  Synthetic
ctggcggcttgaagaatttgg

SEQ ID NO: 22 - DNA, 24 bp, Artificial Sequence
  Synthetic
catgatttccaggttggctttgtc

SEQ ID NO: 23 - DNA, 26 bp, Artificial Sequence
  Synthetic
cgatttgccagctttgaggctcaagg

SEQ ID NO: 24 - DNA, 20 bp, Artificial Sequence
  Synthetic
aggcttgggtgctccacttg

SEQ ID NO: 25 - DNA, 21 bp, Artificial Sequence
  Synthetic
gaccctggtgatgctggaaac

SEQ ID NO: 26 - DNA, 27 bp, Artificial Sequence
  Synthetic
caggtgtaaacctctccactccgagga